European Patent Application EP 4 537 842 A1, published April 16, 2025. Title: 筋萎縮性側索硬化症、パーキンソン病、ハンチントン病、脊髄小脳失調症、老化に関連する変性疾患若しくは神経疾患、脳老化、あるいは脳老化を伴う疾患の予防剤若しくは治療剤. Applicant: 東京医科歯科大学. The sequence listing filed with the application follows.

SEQUENCE LISTING (22 sequences)

SEQ ID NO: 1 - protein, 5 aa, synthetic construct
  REGION 1..5: note = Heavy Chain Complementarity Determination Region 1 of human monoc lonal antibody #129
  REGION 1..5: note = MISC_FEATURE - Inventor:OKAZAWA, Hitoshi
SYAMS

SEQ ID NO: 2 - protein, 17 aa, synthetic construct
  REGION 1..17: note = Heavy Chain Complementarity Determination Region 2 of human monoc lonal antibody #129
DISGSGGSTYYADSVKG

SEQ ID NO: 3 - protein, 6 aa, synthetic construct
  REGION 1..6: note = Heavy Chain Complementarity Determination Region 3 of human monoc lonal antibody #129
GYGMDV

SEQ ID NO: 4 - protein, 11 aa, synthetic construct
  REGION 1..11: note = Light Chain Complementarity Determination Region 1 of human monoc lonal antibody #129
RASQSVTNYLA

SEQ ID NO: 5 - protein, 7 aa, synthetic construct
  REGION 1..7: note = Light Chain Complementarity Determination Region 2 of human monoc lonal antibody #129
GASILET

SEQ ID NO: 6 - protein, 9 aa, synthetic construct
  REGION 1..9: note = Light Chain Complementarity Determination Region 3 of human monoc lonal antibody #129
LQHNSTPLT

SEQ ID NO: 7 - protein, 115 aa, synthetic construct
  REGION 1..115: note = Heavy Chain Variable Region of human monoclonal antibody #129
EVQLLESGGGLVQPGGSLRLSCAASGFTFSSYAMSWVRQAPGKGLEWVSDISGSGGSTYYADSVKGRFTISRDNSKNTLYLQMNSLRAEDTAVYYCARGYGMDVWGQGTMVTVSS

SEQ ID NO: 8 - protein, 107 aa, synthetic construct
  REGION 1..107: note = Light Chain Variable Region of human monoclonal antibody #129
DIQMTQSPSSLSASVGDRVTITCRASQSVTNYLAWYQQKPGKAPKLLIYGASILETGVPSRFSGSGSGTDFTLTINSLQPEDFATYYCLQHNSTPLTFGQGTKLEIK

SEQ ID NO: 9 - protein, 445 aa, synthetic construct
  REGION 1..445: note = Heavy Chain of human monoclonal antibody #129
EVQLLESGGGLVQPGGSLRLSCAASGFTFSSYAMSWVRQAPGKGLEWVSDISGSGGSTYYADSVKGRFTISRDNSKNTLYLQMNSLRAEDTAVYYCARGYGMDVWGQGTMVTVSSASTKGPSVFPLAPSSKSTSGGTAALGCLVKDYFPEPVTVSWNSGALTSGVHTFPAVLQSSGLYSLSSVVTVPSSSLGTQTYICNVNHKPSNTKVDKKVEPKSCDKTHTCPPCPAPELLGGPSVFLFPPKPKDTLMISRTPEVTCVVVDVSHEDPEVKFNWYVDGVEVHNAKTKPREEQYNSTYRVVSVLTVLHQDWLNGKEYKCKVSNKALPAPIEKTISKAKGQPREPQVYTLPPSREEMTKNQVSLTCLVKGFYPSDIAVEWESNGQPENNYKTTPPVLDSDGSFFLYSKLTVDKSRWQQGNVFSCSVMHEALHNHYTQKSLSLSPGK

SEQ ID NO: 10 - protein, 213 aa, synthetic construct
  REGION 1..213: note = Light Chain of human monoclonal antibody #129
DIQMTQSPSSLSASVGDRVTITCRASQSVTNYLAWYQQKPGKAPKLLIYGASILETGVPSRFSGSGSGTDFTLTINSLQPEDFATYYCLQHNSTPLTFGQGTKLEIKTVAAPSVFIFPPSDEQLKSGTASVVCLLNNFYPREAKVQWKVDNALQSGNSQESVTEQDSKDSTYSLSSTLTLSKADYEKHKVYACEVTHQGLSSPVTKSFNRGEC

SEQ ID NO: 11 - DNA, 25 bp, synthetic construct
  misc_feature 1..25: note = primer 1
  source 1..25: mol_type = other DNA
atatgctctcactgtatggtattgc

SEQ ID NO: 12 - DNA, 25 bp, synthetic construct
  misc_feature 1..25: note = primer 2
  source 1..25: mol_type = other DNA
tccagatgagcttagaagattagaa

SEQ ID NO: 13 - DNA, 25 bp, synthetic construct
  misc_feature 1..25: note = primer 3
  source 1..25: mol_type = other DNA
tggattttatttatgtctgaatgtg

SEQ ID NO: 14 - DNA, 25 bp, synthetic construct
  misc_feature 1..25: note = primer 4
  source 1..25: mol_type = other DNA
ataagcaacttcacaaggcatctta

SEQ ID NO: 15 - DNA, 25 bp, synthetic construct
  misc_feature 1..25: note = primer 5
  source 1..25: mol_type = other DNA
acagttgggtgtgatagcaggtact

SEQ ID NO: 16 - DNA, 25 bp, synthetic construct
  misc_feature 1..25: note = primer 6
  source 1..25: mol_type = other DNA
tcgagaattacaggaatgtatcatc

SEQ ID NO: 17 - protein, 9 aa, synthetic construct
  REGION 1..9: note = Light Chain Complementarity Determination Region 3 of human monoc lonal antibody #129-L1
LQHNANPLT

SEQ ID NO: 18 - protein, 106 aa, synthetic construct
  REGION 1..106: note = Light Chain Variable Region of human monoclonal antibody #129-L1
DIQMTQSPSSLSASVGDRVTITCRASQSVTNYLAWYQQKPGKAPKLLIYGASILETGVPSRFSGSGSGTDFTLTINSLQPEDFATYYCLQHANPLTFGQGTKLEIK

SEQ ID NO: 19 - protein, 212 aa, synthetic construct
  REGION 1..212: note = Light Chain of human monoclonal antibody #129-L1
DIQMTQSPSSLSASVGDRVTITCRASQSVTNYLAWYQQKPGKAPKLLIYGASILETGVPSRFSGSGSGTDFTLTINSLQPEDFATYYCLQHANPLTFGQGTKLEIKTVAAPSVFIFPPSDEQLKSGTASVVCLLNNFYPREAKVQWKVDNALQSGNSQESVTEQDSKDSTYSLSSTLTLSKADYEKHKVYACEVTHQGLSSPVTKSFNRGEC

SEQ ID NO: 20 - protein, 9 aa, synthetic construct
  REGION 1..9: note = Light Chain Complementarity Determination Region 3 of human monoc lonal antibody #129-L2
LQHASTPLT

SEQ ID NO: 21 - protein, 107 aa, synthetic construct
  REGION 1..107: note = Light Chain Variable Region of human monoclonal antibody #129-L2
DIQMTQSPSSLSASVGDRVTITCRASQSVTNYLAWYQQKPGKAPKLLIYGASILETGVPSRFSGSGSGTDFTLTINSLQPEDFATYYCLQHASTPLTFGQGTKLEIK

SEQ ID NO: 22 - protein, 213 aa, synthetic construct
  REGION 1..213: note = Light Chain of human monoclonal antibody #129-L2
DIQMTQSPSSLSASVGDRVTITCRASQSVTNYLAWYQQKPGKAPKLLIYGASILETGVPSRFSGSGSGTDFTLTINSLQPEDFATYYCLQHASTPLTFGQGTKLEIKTVAAPSVFIFPPSDEQLKSGTASVVCLLNNFYPREAKVQWKVDNALQSGNSQESVTEQDSKDSTYSLSSTLTLSKADYEKHKVYACEVTHQGLSSPVTKSFNRGEC